European Patent Specification EP 3 335 722 B1, published July 26, 2023. Title: Compositions for Intercelluar Delivery Comprising Peptide derived from Adenovirus Protein VI and Pharmaceutical Compositions for Treating Cancer Comprising the Same. Applicant: Industry-university Cooperation Foundation Hanyang University. The sequence listing filed with the application follows.

SEQUENCE LISTING (11 sequences)

SEQ ID NO: 1 - protein, 13 aa, VI
SWGSLWSGIKNFG

SEQ ID NO: 2 - protein, 22 aa, Artificial Sequence
  VI-9R
SWGSLWSGIKNFGRRRRRRRRR

SEQ ID NO: 3 - protein, 15 aa, Artificial Sequence
  mVI
AFSWGSLWSGIKNFG

SEQ ID NO: 4 - protein, 24 aa, Artificial Sequence
  mVI-TAT
AFSWGSLWSGIKNFGRKKRRQRRR

SEQ ID NO: 5 - protein, 28 aa, Artificial Sequence
  mVI-TAT-A
AFSWGSLWSGIKNFGRKKRRQRRRALAE

SEQ ID NO: 6 - protein, 31 aa, Artificial Sequence
  mVI-G-TAT-A
AFSWGSLWSGIKNFGFLGRKKRRQRRRALAE

SEQ ID NO: 7 - protein, 28 aa, Artificial Sequence
  mVI-A-TAT
AFSWGSLWSGIKNFGALAERKKRRQRRR

SEQ ID NO: 8 - protein, 31 aa, Artificial Sequence
  mVI-G-A-TAT
AFSWGSLWSGIKNFGFLGALAERKKRRQRRR

SEQ ID NO: 9 - protein, 11 aa, Artificial Sequence
  TAT
YGRKKRRQRRR

SEQ ID NO: 10 - protein, 14 aa, Artificial Sequence
  NLS
PKKKRKVPKKKRKV

SEQ ID NO: 11 - protein, 62 aa, Artificial Sequence
  mVI-G-A-TAT dimer
AFSWGSLWSGIKNFGFLGALAERKKRRQRRRAFSWGSLWSGIKNFGFLGALAERKKRRQRRR